European Patent Specification EP 3 294 766 B1, published August 9, 2023. Title: Humanized antibody or fragment thereof specific for CD3. Applicant: Miltenyi Biotec GmbH. The sequence listing filed with the application follows.

SEQUENCE LISTING (34 sequences)

SEQ ID NO: 1 - protein, 8 aa, Artificial Sequence
  CDR1 of heavy chain variable domain of anti-CD3
GYTFTRYT

SEQ ID NO: 2 - protein, 8 aa, Artificial Sequence
  CDR2 of heavy chain variable domain of anti-CD3
INPSRGYT

SEQ ID NO: 3 - protein, 12 aa, Artificial Sequence
  CDR3 of heavy chain variable domain of anti-CD3
ARYYDDHYSLDY

SEQ ID NO: 4 - protein, 5 aa, Artificial Sequence
  CDR1 of light chain variable domain of anti-CD3
SSVSY

SEQ ID NO: 5 - protein, 3 aa, Artificial Sequence
  CDR2 of light chain variable domain of anti-CD3
DTS

SEQ ID NO: 6 - protein, 9 aa, Artificial Sequence
  CDR3 of light chain variable domain of anti-CD3
QQWSSNPFT

SEQ ID NO: 7 - protein, 8 aa, Artificial Sequence
  CDR1 of heavy chain variable domain of anti-CD28
GFSLTSYG

SEQ ID NO: 8 - protein, 7 aa, Artificial Sequence
  CDR2 of heavy chain variable domain of anti-CD28
IWAGGST

SEQ ID NO: 9 - protein, 17 aa, Artificial Sequence
  CDR3 of heavy chain variable domain of anti-CD28
ARDKRAPGKLYYGYPDY

SEQ ID NO: 10 - protein, 10 aa, Artificial Sequence
  CDR1 of light chain variable domain of anti-CD28
ESVEYYVTSL

SEQ ID NO: 11 - protein, 3 aa, Artificial Sequence
  CDR2 of light chain variable domain of anti-CD28
AAS

SEQ ID NO: 12 - protein, 9 aa, Artificial Sequence
  CDR3 of light chain variable domain of anti-CD28
QQTRKVPST

SEQ ID NO: 13 - protein, 119 aa, Mus musculus [sequence omitted]

SEQ ID NO: 14 - protein, 106 aa, Mus musculus [sequence omitted]

SEQ ID NO: 15 - protein, 119 aa, Artificial Sequence
  heavy chain variable domain of anti-chCD3_mut
QVQLQQSGAELARPGASVKMSCKASGYTFTRYTMHWVKQRPGQGLEWIGYINPSRGYTNYNQKFKDKATLTTDKSSSTAYMQLSSLTSEDSAVYYCARYYDDHYSLDYWGQGTTLTVSS

SEQ ID NO: 16 - protein, 119 aa, Artificial Sequence
  heavy chain variable domain of anti-huCD3_mut
QVQLVQSGGGVVQPGRSLRLSCKASGYTFTRYTMHWVRQAPGKGLEWIGYINPSRGYTNYNQKVKDRFTISRDNSKNTAFLQMDSLRPEDTGVYFCARYYDDHYSLDYWGQGTPVTVSS

SEQ ID NO: 17 - protein, 106 aa, Artificial Sequence [sequence omitted]

SEQ ID NO: 18 - protein, 123 aa, Mus musculus
  heavy chain variable domain of anti-chCD28
QVQLKESGPGLVAPSQSLSITCTVSGFSLTSYGVHWVRQPPGKGLEWLGVIWAGGSTNYNSALMSRLSISKDNSKSQVFLKMNSLQTDDTAMYYCARDKRAPGKLYYGYPDYWGQGTTLTVSS

SEQ ID NO: 19 - protein, 111 aa, Mus musculus
  light chain variable domain of anti-chCD28
DIVLTQSPASLAVSLGQRATISCRASESVEYYVTSLMQWYQQKPGQPPKLLIYAASNVESGVPARFSGSGSGTDFSLNIHPVEEDDIAMYFCQQTRKVPSTFGGGTKLEIK

SEQ ID NO: 20 - protein, 123 aa, Artificial Sequence
  heavy chain variable domain of anti-huCD28_v1
QVQLQESGPGLVKPSETLSLTCTVSGFSLTSYGVHWVRQPPGKGLEWLGVIWAGGSTNYNSALMSRLTISKDTSKNQVSLKLSSVTAADTAVYYCARDKRAPGKLYYGYPDYWGQGTTLTVSS

SEQ ID NO: 21 - protein, 111 aa, Artificial Sequence
  light chain variable domain of anti-huCD28_v1
DIVMTQSPDSLAVSLGERATINCRASESVEYYVTSLMQWYQQKPGQPPKLLIYAASNVESGVPDRFSGSGSGTDFTLTISSLQAEDVAVYYCQQTRKVPSTFGGGTKLEIK

SEQ ID NO: 22 - protein, 123 aa, Artificial Sequence
  heavy chain variable domain of anti-huCD28_v2
QVQLQESGPGLVKPSETLSLTCTVSGFSLTSYGVHWVRQPPGKGLEWIGVIWAGGSTNYNPSLKSRVTISKDTSKNQFSLKLSSVTAADTAVYYCARDKRAPGKLYYGYPDYWGQGTTLTVSS

SEQ ID NO: 23 - protein, 111 aa, Artificial Sequence
  light chain variable domain of anti-huCD28_v2
DIVMTQSPDSLAVSLGERATINCKSSESVEYYVTSLLQWYQQKPGQPPKLLIYAASNRESGVPDRFSGSGSGTDFTLTISSLQAEDVAVYYCQQTRKVPSTFGGGTKLEIK

SEQ ID NO: 24 - protein, 123 aa, Artificial Sequence
  heavy chain variable domain of anti-huCD28_v3
QVQLQESGPGLVKPSETLSLTCTVSGFSLTSYGVHWIRQPPGKGLEWLGVIWAGGSTNYNSSLKSRVTISKDTSKNQVFLKLSSVTADDTAVYYCARDKRAPGKLYYGYPDYWGQGTTLTVSS

SEQ ID NO: 25 - protein, 111 aa, Artificial Sequence
  light chain variable domain of anti-huCD28_v3 and of anti-huCD28_v4
DIVMTQSPDSLAVSLGERATINCRASESVEYYVTSLMQWYQQKPGQPPKLLIYAASNVESGVPARFSGSGSGTDFTLTISPLQAEDVAVYYCQQTRKVPSTFGGGTKLEIK

SEQ ID NO: 26 - protein, 123 aa, Artificial Sequence
  heavy chain variable domain of anti-huCD28_v4
QVQLQESGPGLVKPSETLSLTCTVSGFSLTSYGVHWIRQPPGKGLEWLGVIWAGGSTNYNSSLKSRVTISKDTSKNQVSLKLSSVTAADTAVYYCARDKRAPGKLYYGYPDYWGQGTTLTVSS

SEQ ID NO: 27 - protein, 97 aa, Homo sapiens
  protein sequence of IGHV4-4*08 allele according to IMGT
QVQLQESGPGLVKPSETLSLTCTVSGGSISSYYWSWIRQPPGKGLEWIGYIYTSGSTNYNPSLKSRVTISVDTSKNQFSLKLSSVTAADTAVYYCAR

SEQ ID NO: 28 - protein, 101 aa, Homo sapiens
  protein sequence of IGKV4-1*01 allele according to IMGT
DIVMTQSPDSLAVSLGERATINCKSSQSVLYSSNNKNYLAWYQQKPGQPPKLLIYWASTRESGVPDRFSGSGSGTDFTLTISSLQAEDVAVYYCQQYYSTP

SEQ ID NO: 29 - protein, 123 aa, Artificial Sequence; identical to SEQ ID NO: 22
  anti-CD28graft VH_final_IMGT

SEQ ID NO: 30 - protein, 111 aa, Artificial Sequence; identical to SEQ ID NO: 23
  anti-CD28graft VL_final_IMGT

SEQ ID NO: 31 - protein, 103 aa, Homo sapiens
  human IgG1 heavy chain constant region CH1
ASTKGPSVFPLAPSSKSTSGGTAALGCLVKDYFPEPVTVSWNSGALTSGVHTFPAVLQSSGLYSLSSVVTVPSSSLGTQTYICNVNHKPSNTKVDKKVEPKSC

SEQ ID NO: 32 - protein, 107 aa, Homo sapiens [sequence omitted]

SEQ ID NO: 33 - protein, 15 aa, Homo sapiens
  protein sequence of IGHJ4*01 allele according to IMGT
YFDYWGQGTLVTVSS

SEQ ID NO: 34 - protein, 12 aa, Homo sapiens
  protein sequence of IGKJ4*01 allele according to IMGT
LTFGGGTKVEIK